European Patent Specification EP 4 005 590 B1, published December 4, 2024. Title: METHODS AND COMPOSITIONS FOR MODULATING THE IMMUNE SYSTEM WITH ARGINASE I. Applicant: BIO-CANCER TREATMENT INTERNATIONAL LIMITED. Application EP 21203466.4. The sequence listing filed with the application follows.

SEQUENCE LISTING (32 sequences)

SEQ ID NO: 1 - protein, 322 aa, Homo sapiens
MSAKSRTIGIIGAPFSKGQPRGGVEEGPTVLRKAGLLEKLKEQECDVKDYGDLPFADIPNDSPFQIVKNPRSVGKASEQLAGKVAEVKKNGRISLVLGGDHSLAIGSISGHARVHPDLGVIWVDAHTDINTPLTTTSGNLHGQPVSFLLKELKGKIPDVPGFSWVTPCISAKDIVYIGLRDVDPGEHYILKTLGIKYFSMTEVDRLGIGKVMEETLSYLLGRKKRPIHLSFDVDGLDPSFTPATGTPVVGGLTYREGLYITEEIYKTGLLSGLDIMEVNPSLGKTPEEVTRTVNTAVAITLACFGLAREGNHKPIDYLNPPK

SEQ ID NO: 2 - protein, 322 aa, Artificial Sequence
  Description of Artificial Sequence: Synthetic polypeptide
MSAKSRTIGIIGAPFSKGQPRGGVEEGPTVLRKAGLLEKLKEQECDVKDYGDLPFADIPNDSPFQIVKNPRSVGKASEQLAGKVAEVKKNGRISLVLGGDHSLAIGSISGHARVHPDLGVIWVDAHTDINTPLTTTSGNLHGQPVSFLLKELKGKIPDVPGFSWVTPCISAKDIVYIGLRDVDPGEHYILKTLGIKYFSMTEVDRLGIGKVMEETLSYLLGRKKRPIHLSFDVDGLDPSFTPATGTPVVGGLTYREGLYITEEIYKTGLLSGLDIMEVNPSLGKTPEEVTRTVNTAVAITLAAFGLAREGNHKPIDYLNPPK

SEQ ID NO: 3 - protein, 322 aa, Artificial Sequence
  Description of Artificial Sequence: Synthetic polypeptide
MSAKSRTIGIIGAPFSKGQPRGGVEEGPTVLRKAGLLEKLKEQECDVKDYGDLPFADIPNDSPFQIVKNPRSVGKASEQLAGKVAEVKKNGRISLVLGGDHSLAIGSISGHARVHPDLGVIWVDAHTDINTPLTTTSGNLHGQPVSFLLKELKGKIPDVPGFSWVTPAISAKDIVYIGLRDVDPGEHYILKTLGIKYFSMTEVDRLGIGKVMEETLSYLLGRKKRPIHLSFDVDGLDPSFTPATGTPVVGGLTYREGLYITEEIYKTGLLSGLDIMEVNPSLGKTPEEVTRTVNTAVAITLACFGLAREGNHKPIDYLNPPK

SEQ ID NO: 4 - protein, 322 aa, Artificial Sequence
  Description of Artificial Sequence: Synthetic polypeptide
MSAKSRTIGIIGAPFSKGQPRGGVEEGPTVLRKAGLLEKLKEQEADVKDYGDLPFADIPNDSPFQIVKNPRSVGKASEQLAGKVAEVKKNGRISLVLGGDHSLAIGSISGHARVHPDLGVIWVDAHTDINTPLTTTSGNLHGQPVSFLLKELKGKIPDVPGFSWVTPCISAKDIVYIGLRDVDPGEHYILKTLGIKYFSMTEVDRLGIGKVMEETLSYLLGRKKRPIHLSFDVDGLDPSFTPATGTPVVGGLTYREGLYITEEIYKTGLLSGLDIMEVNPSLGKTPEEVTRTVNTAVAITLACFGLAREGNHKPIDYLNPPK

SEQ ID NO: 5 - protein, 322 aa, Artificial Sequence
  Description of Artificial Sequence: Synthetic polypeptide
MSAKSRTIGIIGAPFSKGQPRGGVEEGPTVLRKAGLLEKLKEQECDVKDYGDLPFADIPNDSPFQIVKNPRSVGKASEQLAGKVAEVKKNGRISLVLGGDHSLAIGSISGHARVHPDLGVIWVDAHTDINTPLTTTSGNLHGQPVSFLLKELKGKIPDVPGFSWVTPAISAKDIVYIGLRDVDPGEHYILKTLGIKYFSMTEVDRLGIGKVMEETLSYLLGRKKRPIHLSFDVDGLDPSFTPATGTPVVGGLTYREGLYITEEIYKTGLLSGLDIMEVNPSLGKTPEEVTRTVNTAVAITLAAFGLAREGNHKPIDYLNPPK

SEQ ID NO: 6 - protein, 322 aa, Artificial Sequence
  Description of Artificial Sequence: Synthetic polypeptide
MSAKSRTIGIIGAPFSKGQPRGGVEEGPTVLRKAGLLEKLKEQEADVKDYGDLPFADIPNDSPFQIVKNPRSVGKASEQLAGKVAEVKKNGRISLVLGGDHSLAIGSISGHARVHPDLGVIWVDAHTDINTPLTTTSGNLHGQPVSFLLKELKGKIPDVPGFSWVTPCISAKDIVYIGLRDVDPGEHYILKTLGIKYFSMTEVDRLGIGKVMEETLSYLLGRKKRPIHLSFDVDGLDPSFTPATGTPVVGGLTYREGLYITEEIYKTGLLSGLDIMEVNPSLGKTPEEVTRTVNTAVAITLAAFGLAREGNHKPIDYLNPPK

SEQ ID NO: 7 - protein, 322 aa, Artificial Sequence
  Description of Artificial Sequence: Synthetic polypeptide
MSAKSRTIGIIGAPFSKGQPRGGVEEGPTVLRKAGLLEKLKEQEADVKDYGDLPFADIPNDSPFQIVKNPRSVGKASEQLAGKVAEVKKNGRISLVLGGDHSLAIGSISGHARVHPDLGVIWVDAHTDINTPLTTTSGNLHGQPVSFLLKELKGKIPDVPGFSWVTPAISAKDIVYIGLRDVDPGEHYILKTLGIKYFSMTEVDRLGIGKVMEETLSYLLGRKKRPIHLSFDVDGLDPSFTPATGTPVVGGLTYREGLYITEEIYKTGLLSGLDIMEVNPSLGKTPEEVTRTVNTAVAITLACFGLAREGNHKPIDYLNPPK

SEQ ID NO: 8 - protein, 322 aa, Artificial Sequence
  Description of Artificial Sequence: Synthetic polypeptide
MSAKSRTIGIIGAPFSKGQPRGGVEEGPTVLRKAGLLEKLKEQEADVKDYGDLPFADIPNDSPFQIVKNPRSVGKASEQLAGKVAEVKKNGRISLVLGGDHSLAIGSISGHARVHPDLGVIWVDAHTDINTPLTTTSGNLHGQPVSFLLKELKGKIPDVPGFSWVTPAISAKDIVYIGLRDVDPGEHYILKTLGIKYFSMTEVDRLGIGKVMEETLSYLLGRKKRPIHLSFDVDGLDPSFTPATGTPVVGGLTYREGLYITEEIYKTGLLSGLDIMEVNPSLGKTPEEVTRTVNTAVAITLAAFGLAREGNHKPIDYLNPPK

SEQ ID NO: 9 - protein, 329 aa, Artificial Sequence
  Description of Artificial Sequence: Synthetic polypeptide
MHHHHHHMSAKSRTIGIIGAPFSKGQPRGGVEEGPTVLRKAGLLEKLKEQECDVKDYGDLPFADIPNDSPFQIVKNPRSVGKASEQLAGKVAEVKKNGRISLVLGGDHSLAIGSISGHARVHPDLGVIWVDAHTDINTPLTTTSGNLHGQPVSFLLKELKGKIPDVPGFSWVTPCISAKDIVYIGLRDVDPGEHYILKTLGIKYFSMTEVDRLGIGKVMEETLSYLLGRKKRPIHLSFDVDGLDPSFTPATGTPVVGGLTYREGLYITEEIYKTGLLSGLDIMEVNPSLGKTPEEVTRTVNTAVAITLACFGLAREGNHKPIDYLNPPK

SEQ ID NO: 10 - protein, 329 aa, Artificial Sequence
  Description of Artificial Sequence: Synthetic polypeptide
MHHHHHHMSAKSRTIGIIGAPFSKGQPRGGVEEGPTVLRKAGLLEKLKEQECDVKDYGDLPFADIPNDSPFQIVKNPRSVGKASEQLAGKVAEVKKNGRISLVLGGDHSLAIGSISGHARVHPDLGVIWVDAHTDINTPLTTTSGNLHGQPVSFLLKELKGKIPDVPGFSWVTPCISAKDIVYIGLRDVDPGEHYILKTLGIKYFSMTEVDRLGIGKVMEETLSYLLGRKKRPIHLSFDVDGLDPSFTPATGTPVVGGLTYREGLYITEEIYKTGLLSGLDIMEVNPSLGKTPEEVTRTVNTAVAITLAAFGLAREGNHKPIDYLNPPK

SEQ ID NO: 11 - protein, 329 aa, Artificial Sequence
  Description of Artificial Sequence: Synthetic polypeptide
MHHHHHHMSAKSRTIGIIGAPFSKGQPRGGVEEGPTVLRKAGLLEKLKEQECDVKDYGDLPFADIPNDSPFQIVKNPRSVGKASEQLAGKVAEVKKNGRISLVLGGDHSLAIGSISGHARVHPDLGVIWVDAHTDINTPLTTTSGNLHGQPVSFLLKELKGKIPDVPGFSWVTPAISAKDIVYIGLRDVDPGEHYILKTLGIKYFSMTEVDRLGIGKVMEETLSYLLGRKKRPIHLSFDVDGLDPSFTPATGTPVVGGLTYREGLYITEEIYKTGLLSGLDIMEVNPSLGKTPEEVTRTVNTAVAITLACFGLAREGNHKPIDYLNPPK

SEQ ID NO: 12 - protein, 329 aa, Artificial Sequence
  Description of Artificial Sequence: Synthetic polypeptide
MHHHHHHMSAKSRTIGIIGAPFSKGQPRGGVEEGPTVLRKAGLLEKLKEQEADVKDYGDLPFADIPNDSPFQIVKNPRSVGKASEQLAGKVAEVKKNGRISLVLGGDHSLAIGSISGHARVHPDLGVIWVDAHTDINTPLTTTSGNLHGQPVSFLLKELKGKIPDVPGFSWVTPCISAKDIVYIGLRDVDPGEHYILKTLGIKYFSMTEVDRLGIGKVMEETLSYLLGRKKRPIHLSFDVDGLDPSFTPATGTPVVGGLTYREGLYITEEIYKTGLLSGLDIMEVNPSLGKTPEEVTRTVNTAVAITLACFGLAREGNHKPIDYLNPPK

SEQ ID NO: 13 - protein, 329 aa, Artificial Sequence
  Description of Artificial Sequence: Synthetic polypeptide
MHHHHHHMSAKSRTIGIIGAPFSKGQPRGGVEEGPTVLRKAGLLEKLKEQECDVKDYGDLPFADIPNDSPFQIVKNPRSVGKASEQLAGKVAEVKKNGRISLVLGGDHSLAIGSISGHARVHPDLGVIWVDAHTDINTPLTTTSGNLHGQPVSFLLKELKGKIPDVPGFSWVTPAISAKDIVYIGLRDVDPGEHYILKTLGIKYFSMTEVDRLGIGKVMEETLSYLLGRKKRPIHLSFDVDGLDPSFTPATGTPVVGGLTYREGLYITEEIYKTGLLSGLDIMEVNPSLGKTPEEVTRTVNTAVAITLAAFGLAREGNHKPIDYLNPPK

SEQ ID NO: 14 - protein, 329 aa, Artificial Sequence
  Description of Artificial Sequence: Synthetic polypeptide
MHHHHHHMSAKSRTIGIIGAPFSKGQPRGGVEEGPTVLRKAGLLEKLKEQEADVKDYGDLPFADIPNDSPFQIVKNPRSVGKASEQLAGKVAEVKKNGRISLVLGGDHSLAIGSISGHARVHPDLGVIWVDAHTDINTPLTTTSGNLHGQPVSFLLKELKGKIPDVPGFSWVTPCISAKDIVYIGLRDVDPGEHYILKTLGIKYFSMTEVDRLGIGKVMEETLSYLLGRKKRPIHLSFDVDGLDPSFTPATGTPVVGGLTYREGLYITEEIYKTGLLSGLDIMEVNPSLGKTPEEVTRTVNTAVAITLAAFGLAREGNHKPIDYLNPPK

SEQ ID NO: 15 - protein, 329 aa, Artificial Sequence
  Description of Artificial Sequence: Synthetic polypeptide
MHHHHHHMSAKSRTIGIIGAPFSKGQPRGGVEEGPTVLRKAGLLEKLKEQEADVKDYGDLPFADIPNDSPFQIVKNPRSVGKASEQLAGKVAEVKKNGRISLVLGGDHSLAIGSISGHARVHPDLGVIWVDAHTDINTPLTTTSGNLHGQPVSFLLKELKGKIPDVPGFSWVTPAISAKDIVYIGLRDVDPGEHYILKTLGIKYFSMTEVDRLGIGKVMEETLSYLLGRKKRPIHLSFDVDGLDPSFTPATGTPVVGGLTYREGLYITEEIYKTGLLSGLDIMEVNPSLGKTPEEVTRTVNTAVAITLACFGLAREGNHKPIDYLNPPK

SEQ ID NO: 16 - protein, 329 aa, Artificial Sequence
  Description of Artificial Sequence: Synthetic polypeptide
MHHHHHHMSAKSRTIGIIGAPFSKGQPRGGVEEGPTVLRKAGLLEKLKEQEADVKDYGDLPFADIPNDSPFQIVKNPRSVGKASEQLAGKVAEVKKNGRISLVLGGDHSLAIGSISGHARVHPDLGVIWVDAHTDINTPLTTTSGNLHGQPVSFLLKELKGKIPDVPGFSWVTPAISAKDIVYIGLRDVDPGEHYILKTLGIKYFSMTEVDRLGIGKVMEETLSYLLGRKKRPIHLSFDVDGLDPSFTPATGTPVVGGLTYREGLYITEEIYKTGLLSGLDIMEVNPSLGKTPEEVTRTVNTAVAITLAAFGLAREGNHKPIDYLNPPK

SEQ ID NO: 17 - DNA, 21 bp, Artificial Sequence
  Description of Artificial Sequence: Synthetic primer
ctcctctactccattcttccc

SEQ ID NO: 18 - DNA, 20 bp, Artificial Sequence
  Description of Artificial Sequence: Synthetic primer
actcccaccaatgaacaaac

SEQ ID NO: 19 - DNA, 25 bp, Artificial Sequence
  Description of Artificial Sequence: Synthetic primer
tcgcgattatcttctatatcttcag

SEQ ID NO: 20 - DNA, 21 bp, Artificial Sequence
  Description of Artificial Sequence: Synthetic primer
gctcgaccagtttagttaccc

SEQ ID NO: 21 - DNA, 39 bp, Artificial Sequence
  Description of Artificial Sequence: Synthetic oligonucleotide
tattagccaatattagccaatattagccaatattagcca

SEQ ID NO: 22 - DNA, 39 bp, Artificial Sequence
  Description of Artificial Sequence: Synthetic oligonucleotide
tggctaatattggctaatattggctaatattggctaata

SEQ ID NO: 23 - DNA, 20 bp, Artificial Sequence
  Description of Artificial Sequence: Synthetic primer
acaccgccaaatttaactgc

SEQ ID NO: 24 - DNA, 20 bp, Artificial Sequence
  Description of Artificial Sequence: Synthetic primer
gtgaagaacccacggtctgt

SEQ ID NO: 25 - DNA, 22 bp, Artificial Sequence
  Description of Artificial Sequence: Synthetic primer
tttctccagtgtagccatcctt

SEQ ID NO: 26 - DNA, 20 bp, Artificial Sequence
  Description of Artificial Sequence: Synthetic primer
ctggattggcaagaagttcc

SEQ ID NO: 27 - DNA, 20 bp, Artificial Sequence
  Description of Artificial Sequence: Synthetic primer
ccctccttctgctctgtgtc

SEQ ID NO: 28 - DNA, 20 bp, Artificial Sequence
  Description of Artificial Sequence: Synthetic primer
tacaccagtccgtccctttc

SEQ ID NO: 29 - DNA, 20 bp, Artificial Sequence
  Description of Artificial Sequence: Synthetic primer
ctggttgtcaggggagtgtt

SEQ ID NO: 30 - DNA, 21 bp, Artificial Sequence
  Description of Artificial Sequence: Synthetic primer
tctgggtacaagatccctgaa

SEQ ID NO: 31 - DNA, 20 bp, Artificial Sequence
  Description of Artificial Sequence: Synthetic primer
cccttctcatctgcatctcc

SEQ ID NO: 32 - DNA, 20 bp, Artificial Sequence
  Description of Artificial Sequence: Synthetic primer
caaacttggtgtggatgtcg